European Patent Specification EP 4 045 658 B1, published September 24, 2025. Title: ASSAYS FOR MEASURING ENZYMATIC ACTIVITIES. Applicant: Agency for Science, Technology and Research. The sequence listing filed with the application follows.

SEQUENCE LISTING (12 sequences)

SEQ ID NO: 1 - DNA, 44 bp, Artificial Sequence
  T7/lacO promoter
taatacgactcactataggggaattgtgagcggataacaattcc

SEQ ID NO: 2 - DNA, 6 bp, Artificial Sequence
  RBS (Ribosome binding site)
aaggag

SEQ ID NO: 3 - DNA, 4137 bp, Artificial Sequence
  Sp Cas9 coding sequence
atggacaagaagtactccattgggctcgatatcggcacaaacagcgtcggctgggccgtcattacggacgagtacaaggtgccgagcaaaaaattcaaagttctgggcaataccgatcgccacagcataaagaagaacctcattggcgccctcctgttcgactccggggaaacggccgaagccacgcggctcaaaagaacagcacggcgcagatatacccgcagaaagaatcggatctgctacctgcaggagatctttagtaatgagatggctaaggtggatgactctttcttccataggctggaggagtcctttttggtggaggaggataaaaagcacgagcgccacccaatctttggcaatatcgtggacgaggtggcgtaccatgaaaagtacccaaccatatatcatctgaggaagaagcttgtagacagtactgataaggctgacttgcggttgatctatctcgcgctggcgcatatgatcaaatttcggggacacttcctcatcgagggggacctgaacccagacaacagcgatgtcgacaaactctttatccaactggttcagacttacaatcagcttttcgaagagaacccgatcaacgcatccggagttgacgccaaagcaatcctgagcgctaggctgtccaaatcccggcggctcgaaaacctcatcgcacagctccctggggagaagaagaacggcctgtttggtaatcttatcgccctgtcactcgggctgacccccaactttaaatctaacttcgacctggccgaagatgccaagcttcaactgagcaaagacacctacgatgatgatctcgacaatctgctggcccagatcggcgaccagtacgcagacctttttttggcggcaaagaacctgtcagacgccattctgctgagtgatattctgcgagtgaacacggagatcaccaaagctccgctgagcgctagtatgatcaagcgctatgatgagcaccaccaagacttgactttgctgaaggcccttgtcagacagcaactgcctgagaagtacaaggaaattttcttcgatcagtctaaaaatggctacgccggatacattgacggcggagcaagccaggaggaattttacaaatttattaagcccatcttggaaaaaatggacggcaccgaggagctgctggtaaagcttaacagagaagatctgttgcgcaaacagcgcactttcgacaatggaagcatcccccaccagattcacctgggcgaactgcacgctatcctcaggcggcaagaggatttctacccctttttgaaagataacagggaaaagattgagaaaatcctcacatttcggataccctactatgtaggccccctcgcccggggaaattccagattcgcgtggatgactcgcaaatcagaagagaccatcactccctggaacttcgaggaagtcgtggataagggggcctctgcccagtccttcatcgaaaggatgactaactttgataaaaatctgcctaacgaaaaggtgcttcctaaacactctctgctgtacgagtacttcacagtttataacgagctcaccaaggtcaaatacgtcacagaagggatgagaaagccagcattcctgtctggagagcagaagaaagctatcgtggacctcctcttcaagacgaaccggaaagttaccgtgaaacagctcaaagaagactatttcaaaaagattgaatgtttcgactctgttgaaatcagcggagtggaggatcgcttcaacgcatccctgggaacgtatcacgatctcctgaaaatcattaaagacaaggacttcctggacaatgaggagaacgaggacattcttgaggacattgtcctcacccttacgttgtttgaagatagggagatgattgaagaacgcttgaaaacttacgctcatctcttcgacgacaaagtcatgaaacagctcaagaggcgccgatatacaggatgggggcggctgtcaagaaaactgatcaatgggatccgagacaagcagagtggaaagacaatcctggattttcttaagtccgatggatttgccaaccggaacttcatgcagttgatccatgatgactctctcacctttaaggaggacatccagaaagcacaagtttctggccagggggacagtcttcacgagcacatcgctaatcttgcaggtagcccagctatcaaaaagggaatactgcagaccgttaaggtcgtggatgaactcgtcaaagtaatgggaaggcataagcccgagaatatcgttatcgagatggcccgagagaaccaaactacccagaagggacagaagaacagtagggaaaggatgaagaggattgaagagggtataaaagaactggggtcccaaatccttaaggaacacccagttgaaaacacccagcttcagaatgagaagctctacctgtactacctgcagaacggcagggacatgtacgtggatcaggaactggacatcaatcggctctccgactacgacgtggatcatatcgtgccccagtcttttctcaaagatgattctattgataataaagtgttgacaagatccgataaaaatagagggaagagtgataacgtcccctcagaagaagttgtcaagaaaatgaaaaattattggcggcagctgctgaacgccaaactgatcacacaacggaagttcgataatctgactaaggctgaacgaggtggcctgtctgagttggataaagccggcttcatcaaaaggcagcttgttgagacacgccagatcaccaagcacgtggcccaaattctcgattcacgcatgaacaccaagtacgatgaaaatgacaaactgattcgagaggtgaaagttattactctgaagtctaagctggtctcagatttcagaaaggactttcagttttataaggtgagagagatcaacaattaccaccatgcgcatgatgcctacctgaatgcagtggtaggcactgcacttatcaaaaaatatcccaagcttgaatctgaatttgtttacggagactataaagtgtacgatgttaggaaaatgatcgcaaagtctgagcaggaaataggcaaggccaccgctaagtacttcttttacagcaatattatgaattttttcaagaccgagattacactggccaatggagagattcggaagcgaccacttatcgaaacaaacggagaaacaggagaaatcgtgtgggacaagggtagggatttcgcgacagtccggaaggtcctgtccatgccgcaggtgaacatcgttaaaaagaccgaagtacagaccggaggcttctccaaggaaagtatcctcccgaaaaggaacagcgacaagctgatcgcacgcaaaaaagattgggaccccaagaaatacggcggattcgattctcctacagtcgcttacagtgtactggttgtggccaaagtggagaaagggaagtctaaaaaactcaaaagcgtcaaggaactgctgggcatcacaatcatggagcgatcaagcttcgaaaaaaaccccatcgactttctcgaggcgaaaggatataaagaggtcaaaaaagacctcatcattaagcttcccaagtactctctctttgagcttgaaaacggccggaaacgaatgctcgctagtgcgggcgagctgcagaaaggtaacgagctggcactgccctctaaatacgttaatttcttgtatctggccagccactatgaaaagctcaaagggtctcccgaagataatgagcagaagcagctgttcgtggaacaacacaaacactaccttgatgagatcatcgagcaaataagcgaattctccaaaagagtgatcctcgccgacgctaacctcgataaggtgctttctgcttacaataagcacagggataagcccatcagggagcaggcagaaaacattatccacttgtttactctgaccaacttgggcgcgcctgcagccttcaagtacttcgacaccaccatagacagaaagcggtacacctctacaaaggaggtcctggacgccacactgattcatcagtcaattacggggctctatgaaacaagaatcgacctctctcagctcggtggagacagcagggctgaccccaagaagaagaggaaggtg

SEQ ID NO: 4 - DNA, 52 bp, Artificial Sequence
  Synthetic terminator sequence (L3S1P52)
tctaactaaaaaggcctcccaaatcggggggccttttttattgataacaaaa

SEQ ID NO: 5 - DNA, 18 bp, Artificial Sequence
  T7 promoter
taatacgactcactatag

SEQ ID NO: 6 - DNA, 26 bp, Artificial Sequence
  gRNA target sequence (protospacer)
tctgacagcagacgtgcactggccag

SEQ ID NO: 7 - DNA, 77 bp, Artificial Sequence
  SpCas9 gRNA scaffold
gttttagagctagaaatagcaagttaaaataaggctagtccgttatcaacttgaaaaagtggcaccgagtcggtgct

SEQ ID NO: 8 - DNA, 48 bp, Artificial Sequence
  T7 terminator
ctagcataaccccttggggcctctaaacgggtcttgaggggttttttg

SEQ ID NO: 9 - DNA, 36 bp, Artificial Sequence
  Target region (a DNA target):
tttatctgacagcagacgtgcactggccagggggat

SEQ ID NO: 10 - DNA, 6416 bp, Artificial Sequence
  Sequence of an exemplary polynucleotide construct
gcgacatcgtataacgttactggtttcacattcaccaccctgaattgactctcttccgggcgctatcatgccataccgcgaaaggttttgcgccattcgatggtgtccgggatctcgacgctctcccttatgcgactcctgcattaggaaattaatacgactcactataggggaattgtgagcggataacaattcccctgtagaaataattttgtttaactttaataaggagatataccatggacaagaagtactccattgggctcgatatcggcacaaacagcgtcggctgggccgtcattacggacgagtacaaggtgccgagcaaaaaattcaaagttctgggcaataccgatcgccacagcataaagaagaacctcattggcgccctcctgttcgactccggggaaacggccgaagccacgcggctcaaaagaacagcacggcgcagatatacccgcagaaagaatcggatctgctacctgcaggagatctttagtaatgagatggctaaggtggatgactctttcttccataggctggaggagtcctttttggtggaggaggataaaaagcacgagcgccacccaatctttggcaatatcgtggacgaggtggcgtaccatgaaaagtacccaaccatatatcatctgaggaagaagcttgtagacagtactgataaggctgacttgcggttgatctatctcgcgctggcgcatatgatcaaatttcggggacacttcctcatcgagggggacctgaacccagacaacagcgatgtcgacaaactctttatccaactggttcagacttacaatcagcttttcgaagagaacccgatcaacgcatccggagttgacgccaaagcaatcctgagcgctaggctgtccaaatcccggcggctcgaaaacctcatcgcacagctccctggggagaagaagaacggcctgtttggtaatcttatcgccctgtcactcgggctgacccccaactttaaatctaacttcgacctggccgaagatgccaagcttcaactgagcaaagacacctacgatgatgatctcgacaatctgctggcccagatcggcgaccagtacgcagacctttttttggcggcaaagaacctgtcagacgccattctgctgagtgatattctgcgagtgaacacggagatcaccaaagctccgctgagcgctagtatgatcaagcgctatgatgagcaccaccaagacttgactttgctgaaggcccttgtcagacagcaactgcctgagaagtacaaggaaattttcttcgatcagtctaaaaatggctacgccggatacattgacggcggagcaagccaggaggaattttacaaatttattaagcccatcttggaaaaaatggacggcaccgaggagctgctggtaaagcttaacagagaagatctgttgcgcaaacagcgcactttcgacaatggaagcatcccccaccagattcacctgggcgaactgcacgctatcctcaggcggcaagaggatttctacccctttttgaaagataacagggaaaagattgagaaaatcctcacatttcggataccctactatgtaggccccctcgcccggggaaattccagattcgcgtggatgactcgcaaatcagaagagaccatcactccctggaacttcgaggaagtcgtggataagggggcctctgcccagtccttcatcgaaaggatgactaactttgataaaaatctgcctaacgaaaaggtgcttcctaaacactctctgctgtacgagtacttcacagtttataacgagctcaccaaggtcaaatacgtcacagaagggatgagaaagccagcattcctgtctggagagcagaagaaagctatcgtggacctcctcttcaagacgaaccggaaagttaccgtgaaacagctcaaagaagactatttcaaaaagattgaatgtttcgactctgttgaaatcagcggagtggaggatcgcttcaacgcatccctgggaacgtatcacgatctcctgaaaatcattaaagacaaggacttcctggacaatgaggagaacgaggacattcttgaggacattgtcctcacccttacgttgtttgaagatagggagatgattgaagaacgcttgaaaacttacgctcatctcttcgacgacaaagtcatgaaacagctcaagaggcgccgatatacaggatgggggcggctgtcaagaaaactgatcaatgggatccgagacaagcagagtggaaagacaatcctggattttcttaagtccgatggatttgccaaccggaacttcatgcagttgatccatgatgactctctcacctttaaggaggacatccagaaagcacaagtttctggccagggggacagtcttcacgagcacatcgctaatcttgcaggtagcccagctatcaaaaagggaatactgcagaccgttaaggtcgtggatgaactcgtcaaagtaatgggaaggcataagcccgagaatatcgttatcgagatggcccgagagaaccaaactacccagaagggacagaagaacagtagggaaaggatgaagaggattgaagagggtataaaagaactggggtcccaaatccttaaggaacacccagttgaaaacacccagcttcagaatgagaagctctacctgtactacctgcagaacggcagggacatgtacgtggatcaggaactggacatcaatcggctctccgactacgacgtggatcatatcgtgccccagtcttttctcaaagatgattctattgataataaagtgttgacaagatccgataaaaatagagggaagagtgataacgtcccctcagaagaagttgtcaagaaaatgaaaaattattggcggcagctgctgaacgccaaactgatcacacaacggaagttcgataatctgactaaggctgaacgaggtggcctgtctgagttggataaagccggcttcatcaaaaggcagcttgttgagacacgccagatcaccaagcacgtggcccaaattctcgattcacgcatgaacaccaagtacgatgaaaatgacaaactgattcgagaggtgaaagttattactctgaagtctaagctggtctcagatttcagaaaggactttcagttttataaggtgagagagatcaacaattaccaccatgcgcatgatgcctacctgaatgcagtggtaggcactgcacttatcaaaaaatatcccaagcttgaatctgaatttgtttacggagactataaagtgtacgatgttaggaaaatgatcgcaaagtctgagcaggaaataggcaaggccaccgctaagtacttcttttacagcaatattatgaattttttcaagaccgagattacactggccaatggagagattcggaagcgaccacttatcgaaacaaacggagaaacaggagaaatcgtgtgggacaagggtagggatttcgcgacagtccggaaggtcctgtccatgccgcaggtgaacatcgttaaaaagaccgaagtacagaccggaggcttctccaaggaaagtatcctcccgaaaaggaacagcgacaagctgatcgcacgcaaaaaagattgggaccccaagaaatacggcggattcgattctcctacagtcgcttacagtgtactggttgtggccaaagtggagaaagggaagtctaaaaaactcaaaagcgtcaaggaactgctgggcatcacaatcatggagcgatcaagcttcgaaaaaaaccccatcgactttctcgaggcgaaaggatataaagaggtcaaaaaagacctcatcattaagcttcccaagtactctctctttgagcttgaaaacggccggaaacgaatgctcgctagtgcgggcgagctgcagaaaggtaacgagctggcactgccctctaaatacgttaatttcttgtatctggccagccactatgaaaagctcaaagggtctcccgaagataatgagcagaagcagctgttcgtggaacaacacaaacactaccttgatgagatcatcgagcaaataagcgaattctccaaaagagtgatcctcgccgacgctaacctcgataaggtgctttctgcttacaataagcacagggataagcccatcagggagcaggcagaaaacattatccacttgtttactctgaccaacttgggcgcgcctgcagccttcaagtacttcgacaccaccatagacagaaagcggtacacctctacaaaggaggtcctggacgccacactgattcatcagtcaattacggggctctatgaaacaagaatcgacctctctcagctcggtggagacagcagggctgaccccaagaagaagaggaaggtggatccaaaaaagaagaggaaggtagatcccaagaaaaaaagaaaagtctcgagcgactacaaagaccatgacggtgattataaagatcatgacatcgattacaaggatgacgatgacaagtgagctttctaactaaaaaggcctcccaaatcggggggccttttttattgataacaaaacgctagcggccgcataatgcttaagtcgaacagaaagtaatcgtattgtacacggccgcataatcgaaattaatacgactcactataggtctgacagcagacgtgcactggccaggttttagagctagaaatagcaagttaaaataaggctagtccgttatcaacttgaaaaagtggcaccgagtcggtgctccgctgagcaataactagcataaccccttggggcctctaaacgggtcttgaggggttttttgttaccctttatctgacagcagacgtgcactggccagggggatggtttgggcctcacgtgacatgtgagcaaaagctgaaacctcaggcatttgagaagcacacggtcacactgcttccggtagtcaataaaccggtaaaccagcaatagacataagcggctatttaacgaccctgccctgaaccgacgaccgggtcgaatttgctttcgaatttctgccattcatccgcttattatcacttattcaggcgtagcaaccaggcgtttaagggcaccaataactgccttaaaaaaattacgccccgccctgccactcatcgcagtactgttgtaattcattaagcattctgccgacatggaagccatcacaaacggcatgatgaacctgaatcgccagcggcatcagcaccttgtcgccttgcgtataatatttgcccatagtgaaaacgggggcgaagaagttgtccatattggccacgtttaaatcaaaactggtgaaactcacccagggattggctgagacgaaaaacatattctcaataaaccctttagggaaataggccaggttttcaccgtaacacgccacatcttgcgaatatatgtgtagaaactgccggaaatcgtcgtggtattcactccagagcgatgaaaacgtttcagtttgctcatggaaaacggtgtaacaagggtgaacactatcccatatcaccagctcaccgtctttcattgccatacggaactccggatgagcattcatcaggcgggcaagaatgtgaataaaggccggataaaacttgtgcttatttttctttacggtctttaaaaaggccgtaatatccagctgaacggtctggttataggtacattgagcaactgactgaaatgcctcaaaatgttctttacgatgccattgggatatatcaacggtggtatatccagtgatttttttctccattttagcttccttagctcctgaaaatctcgataactcaaaaaatacgcccggtagtgatcttatttcattatggtgaaagttggaacctcttacgtgccgatcaacgtctcattttcgccaaaagttggcccagggcttcccggtatcaacagggacaccaggatttatttattctgcgaagtgatcttccgtcacaggtatttattcggcgcaaagtgcgtcgggtgatgctgccaacttactgatttagtgtatgatggtgtttttgaggtgctccagtggcttctgtttctatcagctgtccctcctgttcagctactgacggggtggtgcgtaacggcaaaagcaccgccggacatcagcgctagcggagtgtatactggcttactatgttggcactgatgagggtgtcagtgaagtgcttcatgtggcaggagaaaaaaggctgcaccggtgcgtcagcagaatatgtgatacaggatatattccgcttcctcgctcactgactcgctacgctcggtcgttcgactgcggcgagcggaaatggcttacgaacggggcggagatttcctggaagatgccaggaagatacttaacagggaagtgagagggccgcggcaaagccgtttttccataggctccgcccccctgac

SEQ ID NO: 11 - DNA, 4 bp, Artificial Sequence
  Exemplary 5' PAM site
tttv

SEQ ID NO: 12 - DNA, 6 bp, Artificial Sequence
  An exemplary 3' PAM site
  misc_feature (1)..(2): n is a, c, g, or t
nngrrt